European Patent Specification EP 4 041 286 B1, published July 15, 2026. Title: Recombinant polypeptide for use as a medicine, antiseptic agent, antibacterial agent,. Applicant: MIBMIK. The sequence listing filed with the application follows.

SEQUENCE LISTING (19 sequences)

SEQ ID NO: 1 - protein, 132 aa, Staphylococcus aureus
HAKDASWLTSRKQLQPYGQYHGGGAHYGVDYAMPENSPVYSLTDGTVVQAGWSNYGGGNQVTIKEANSNNYQWYMHNNRLTVSAGDKVKAGDQIAYSGSTGNSTAPHVHFQRMSGGIGNQYAVDPTSYLQSR

SEQ ID NO: 2 - protein, 92 aa, Staphylococcus simulans
WKTNKYGTLYKSESASFTPNTDIITRTTGPFRSMPQSGVLKAGQTIHYDEVMKQDGHVWVGYTGNSGQRIYLPVRTWNKSTNTLGVLWGTIK

SEQ ID NO: 3 - protein, 17 aa, artificial
  LSS- mutated linker
AGYGKAASTVTPTPNTG

SEQ ID NO: 4 - protein, 17 aa, Staphylococcus simulans
AGYGKAGGTVTPTPNTG

SEQ ID NO: 5 - protein, 243 aa, artificial
  Chimeric AA sequence of Chimera A
MGHAKDASWLTSRKQLQPYGQYHGGGAHYGVDYAMPENSPVYSLTDGTVVQAGWSNYGGGNQVTIKEANSNNYQWYMHNNRLTVSAGDKVKAGDQIAYSGSTGNSTAPHVHFQRMSGGIGNQYAVDPTSYLQSRAGYGKAASTVTPTPNTGWKTNKYGTLYKSESASFTPNTDIITRTTGPFRSMPQSGVLKAGQTIHYDEVMKQDGHVWVGYTGNSGQRIYLPVRTWNKSTNTLGVLWGTIK

SEQ ID NO: 6 - DNA, 729 bp, artificial
  Chimera A coding sequence
atgggtcatgcgaaagacgcaagctggttaacaagtcgtaaacaactacaaccatatggacaatatcacggtggtggtgcgcattacggtgtcgactatgcaatgcctgaaaattcaccagtttactcattaactgatggtacagtagtacaagcaggttggagtaactatggtggcggcaatcaagtaacgattaaagaagcgaacagtaataactaccaatggtatatgcataataatcgtttaactgtttcagctggtgataaagtcaaagctggtgaccaaattgcatattcaggtagtacgggtaattcaacagcgcctcacgtacacttccaacgtatgtctggtggcatcggtaatcaatatgcagtagacccaacgtcatacttgcaaagtagagcaggatatggaaaagcagcttctacagtaactccaacgccgaatacaggttggaaaacaaacaaatatggcacactatataaatcagagtcagctagcttcacacctaatacagatataataacaagaacgactggtccatttagaagcatgccgcagtcaggagtcttaaaagcaggtcaaacaattcattatgatgaagtgatgaaacaagacggtcatgtttgggtaggttatacaggtaacagtggccaacgtatttacttgcctgtaagaacatggaataaatctactaatactttaggtgttctttggggaactataaag

SEQ ID NO: 7 - protein, 243 aa, artificial
  AA sequence of Chimera B
MGWKTNKYGTLYKSESASFTPNTDIITRTTGPFRSMPQSGVLKAGQTIHYDEVMKQDGHVWVGYTGNSGQRIYLPVRTWNKSTNTLGVLWGTIKAGYGKAASTVTPTPNTGHAKDASWLTSRKQLQPYGQYHGGGAHYGVDYAMPENSPVYSLTDGTVVQAGWSNYGGGNQVTIKEANSNNYQWYMHNNRLTVSAGDKVKAGDQIAYSGSTGNSTAPHVHFQRMSGGIGNQYAVDPTSYLQSR

SEQ ID NO: 8 - DNA, 729 bp, artificial
  Coding sequence of Chimera B
atgggttggaaaacaaacaaatatggcacactatataaatcagagtcagctagcttcacacctaatacagatataataacaagaacgactggtccatttagaagcatgccgcagtcaggagtcttaaaagcaggtcaaacaattcattatgatgaagtgatgaaacaagacggtcatgtttgggtaggttatacaggtaacagtggccaacgtatttacttgcctgtaagaacatggaataaatctactaatactttaggtgttctttggggaactataaaggcaggatatggaaaagcagcttctacagtaactccaacgccgaatacaggtcatgcgaaagacgcaagctggttaacaagtcgtaaacaactacaaccatatggacaatatcacggtggtggtgcgcattacggtgtcgactatgcaatgcctgaaaattcaccagtttactcattaactgatggtacagtagtacaagcaggttggagtaactatggtggcggcaatcaagtaacgattaaagaagcgaacagtaataactaccaatggtatatgcataataatcgtttaactgtttcagctggtgataaagtcaaagctggtgaccaaattgcatattcaggtagtacgggtaattcaacagcgcctcacgtacacttccaacgtatgtctggtggcatcggtaatcaatatgcagtagacccaacgtcatacttgcaaagtaga

SEQ ID NO: 9 - protein, 16 aa, artificial
  Penatrin
RQIKIWFQNRRMKWKK

SEQ ID NO: 10 - protein, 30 aa, artificial
  CCP2
WEAKLAKALAKALAKHLAKALAKALKACEA

SEQ ID NO: 11 - protein, 22 aa, artificial
  CPP 3
MVTVLFRRLRIRRASGPPRVRV

SEQ ID NO: 12 - protein, 18 aa, artificial
  CPP 4
KLALKLALKALKAALKLA

SEQ ID NO: 13 - protein, 12 aa, artificial
  CPP 5
RRQRRTSKLMKR

SEQ ID NO: 14 - protein, 18 aa, artificial
  CPP 6
LLIILRRRIRKQAHAHSK

SEQ ID NO: 15 - protein, 8 aa, artificial
  poly-arginine
RRRRRRRR

SEQ ID NO: 16 - protein, 13 aa, artificial
  HIV-TAT
GRKKRRQRRRPPQ

SEQ ID NO: 17 - protein, 27 aa, artificial
  CPP 9
GWTLNSAGYLLGKINLKALAALAKKIL

SEQ ID NO: 18 - protein, 21 aa, artificial
  CPP 10
AGYLLGKINLKALAALAKKIL

SEQ ID NO: 19 - protein, 9 aa, artificial
  CPP 11
RKKRRQRRR